European Patent Application EP 4 357 364 A1, published April 24, 2024. Title: 抗体及其应用. Applicant: 合肥天港免疫药物有限公司. Application CN. The sequence listing filed with the application follows.

SEQUENCE LISTING (37 sequences)

SEQ ID NO: 1 - protein, 8 aa, synthetic construct
GFSLTTYG

SEQ ID NO: 2 - protein, 7 aa, synthetic construct
IWTDGTT

SEQ ID NO: 3 - protein, 13 aa, synthetic construct
VRKGHGYYYAMDY

SEQ ID NO: 4 - protein, 7 aa, synthetic construct
SSVSSSY

SEQ ID NO: 5 - skipped

SEQ ID NO: 6 - protein, 9 aa, synthetic construct
HQYHRSPFT

SEQ ID NO: 7 - protein, 119 aa, synthetic construct
QVQLKQSGPGLVQPSQSLSITCIVSGFSLTTYGVHWVRQSPGKGLEWLGMIWTDGTTDYNAAFISRLSINKDNSKSQVFLKMNSLQADDTGIYYCVRKGHGYYYAMDYWGQGTSVTVSS

SEQ ID NO: 8 - protein, 108 aa, synthetic construct
QILLTQSPAILSASLGERVTMTCTASSSVSSSYLHWYQQKPGSSPKLWIYSTSNLASGVPARFSGGGSGTSYSLTVSNMEAEDAATYYCHQYHRSPFTFGSGTKLEIK

SEQ ID NO: 9 - protein, 449 aa, synthetic construct
QVQLKQSGPGLVQPSQSLSITCIVSGFSLTTYGVHWVRQSPGKGLEWLGMIWTDGTTDYNAAFISRLSINKDNSKSQVFLKMNSLQADDTGIYYCVRKGHGYYYAMDYWGQGTSVTVSSAKTTAPSVYPLAPVCGDTTGSSVTLGCLVKGYFPEPVTLTWNSGSLSSGVHTFPAVLQSDLYTLSSSVTVTSSTWPSQSITCNVAHPASSTKVDKKIEPRGPTIKPCPPCKCPAPNLLGGPSVFIFPPKIKDVLMISLSPIVTCVVVDVSEDDPDVQISWFVNNVEVHTAQTQTHREDYNSTLRVVSALPIQHQDWMSGKEFKCKVNNKDLPAPIERTISKPKGSVRAPQVYVLPPPEEEMTKKQVTLTCMVTDFMPEDIYVEWTNNGKTELNYKNTEPVLDSDGSYFMYSKLRVEKKNWVERNSYSCSVVHEGLHNHHTTKSFSRTPGK

SEQ ID NO: 10 - protein, 215 aa, synthetic construct
QILLTQSPAILSASLGERVTMTCTASSSVSSSYLHWYQQKPGSSPKLWIYSTSNLASGVPARFSGGGSGTSYSLTVSNMEAEDAATYYCHQYHRSPFTFGSGTKLEIKRADAAPTVSIFPPSSEQLTSGGASVVCFLNNFYPKDINVKWKIDGSERQNGVLNSWTDQDSKDSTYSMSSTLTLTKDEYERHNSYTCEATHKTSTSPIVKSFNRNEC

SEQ ID NO: 11 - protein, 383 aa, synthetic construct
MGLGPVFLLLAGIFPFAPPGAAAEPHSLRYNLTVLSWDGSVQSGFLTEVHLDGQPFLRCDRQKCRAKPQGQWAEDVLGNKTWDRETRDLTGNGKDLRMTLAHIKDQKEGLHSLQEIRVCEIHEDNSTRSSQHFYYDGELFLSQNLETKEWTMPQSSRAQTLAMNVRNFLKEDAMKTKTHYHAMHADCLQELRRYLKSGVVLRRTVPPMVNVTRSEASEGNITVTCRASGFYPWNITLSWRQDGVSLSHDTQQWGDVLPDGNGTYQTWVATRICQGEEQRFTCYMEHSGNHSTHPVPSGKVLVLQSHWQTFHVSAVAAAAIFVIIIFYVRCCKKKTSAAEGPELVSLQVLDQHPVGTSDHRDATQLGFQPLMSDLGSTGSTEGA

SEQ ID NO: 12 - DNA, 1347 bp, synthetic construct
  source 1..1347: mol_type = other DNA
caggtgcagttgaaacagtctggtcctgggcttgtacagccatctcagtctctgtctattacctgtattgtgtccgggttttcactgacaacttacggcgtgcactgggttaggcagtctccaggtaagggcttggagtggcttggcatgatttggactgatgggaccacagactacaacgctgctttcatcagtcgcctgtccatcaataaggacaactctaaaagccaggtatttctgaagatgaacagcttgcaagctgacgacaccggaatttactactgcgtgcggaagggccatgggtactactatgccatggattattggggtcagggcaccagcgtcacagtatcctctgccaaaacaactgcaccatctgtttatccactggcccccgtttgcggggataccactggtagctctgtcaccctcggctgtctggtcaaaggatatttccccgagcctgtgacacttacctggaattcaggcagcttgtcctccggcgtgcatactttccctgcagtcctgcagtcagatctgtacaccctcagctcatctgtgactgtcacaagttctacctggccatcccagagtattacatgcaacgtggcccacccagcaagttcaacaaaagttgacaagaagattgagccaagaggccctactatcaagccctgtcccccctgtaagtgtcctgcacccaatctgctggggggcccatctgtgtttattttccccccaaagattaaggacgtcctcatgattagcctgtccccaatcgtgacatgtgtggtggtggatgtttctgaggacgacccagacgtacagatctcttggttcgtgaacaatgtcgaggtgcatacagcccagacccagacccatcgggaagactacaactctacattgagagtggtgtccgctttgcccatccagcatcaggactggatgtccggcaaggagtttaaatgtaaggtcaacaacaaggacctgcccgctccaatagagagaactatctcaaagcctaaaggtagtgttcgagccccccaggtatacgtactgccaccccctgaggaggagatgaccaagaagcaggtgacactgacctgcatggtgacagacttcatgccagaagacatttatgtcgaatggactaataatggcaagaccgaactgaattataaaaataccgaaccagtgctggactccgacgggtcctatttcatgtactctaagctccgtgtcgaaaagaagaactgggtggaacgaaactcttactcctgcagtgttgtgcacgaggggcttcacaaccatcatacaaccaagtccttctccaggacacctgggaag

SEQ ID NO: 13 - DNA, 645 bp, synthetic construct
  source 1..645: mol_type = other DNA
cagatcctgttgacccaaagtccagctattctttcagcctctttgggcgaacgtgtgactatgacctgcactgcttccagcagcgtgtccagctcctacttgcactggtatcagcagaagcctggttcatcccctaagctgtggatctattccacctccaacctcgcttcaggagtgcctgccagattttccggaggcggaagtggcacttcctactcacttacagtcagcaacatggaggcagaggacgcagctacctactactgccatcagtatcataggtcccctttcactttcgggtccggtaccaagctcgagatcaaacgagctgatgctgcccccactgtctctatttttcctcctagtagtgagcagctgacatctggaggcgcctccgtggtgtgcttcctgaataacttttaccctaaggacatcaatgtgaagtggaagatcgacgggagtgagaggcagaatggcgtactgaattcctggactgatcaggactctaaagatagcacctatagcatgtcctccaccctcacactgacaaaggacgaatacgaacggcataactcctatacatgtgaggctacccacaagacatccacctcaccaatcgtcaagagcttcaaccggaatgagtgt

SEQ ID NO: 14 - protein, 330 aa, synthetic construct
AKTTAPSVYPLAPVCGDTTGSSVTLGCLVKGYFPEPVTLTWNSGSLSSGVHTFPAVLQSDLYTLSSSVTVTSSTWPSQSITCNVAHPASSTKVDKKIEPRGPTIKPCPPCKCPAPNLLGGPSVFIFPPKIKDVLMISLSPIVTCVVVDVSEDDPDVQISWFVNNVEVHTAQTQTHREDYNSTLRVVSALPIQHQDWMSGKEFKCKVNNKDLPAPIERTISKPKGSVRAPQVYVLPPPEEEMTKKQVTLTCMVTDFMPEDIYVEWTNNGKTELNYKNTEPVLDSDGSYFMYSKLRVEKKNWVERNSYSCSVVHEGLHNHHTTKSFSRTPGK

SEQ ID NO: 15 - DNA, 24 bp, synthetic construct
  source 1..24: mol_type = other DNA
gggttttcactgacaacttacggc

SEQ ID NO: 16 - DNA, 21 bp, synthetic construct
  source 1..21: mol_type = other DNA
atttggactgatgggaccaca

SEQ ID NO: 17 - DNA, 39 bp, synthetic construct
  source 1..39: mol_type = other DNA
gtgcggaagggccatgggtactactatgccatggattat

SEQ ID NO: 18 - DNA, 21 bp, synthetic construct
  source 1..21: mol_type = other DNA
agcagcgtgtccagctcctac

SEQ ID NO: 19 - skipped

SEQ ID NO: 20 - DNA, 27 bp, synthetic construct
  source 1..27: mol_type = other DNA
catcagtatcataggtcccctttcact

SEQ ID NO: 21 - DNA, 357 bp, synthetic construct
  source 1..357: mol_type = other DNA
caggtgcagttgaaacagtctggtcctgggcttgtacagccatctcagtctctgtctattacctgtattgtgtccgggttttcactgacaacttacggcgtgcactgggttaggcagtctccaggtaagggcttggagtggcttggcatgatttggactgatgggaccacagactacaacgctgctttcatcagtcgcctgtccatcaataaggacaactctaaaagccaggtatttctgaagatgaacagcttgcaagctgacgacaccggaatttactactgcgtgcggaagggccatgggtactactatgccatggattattggggtcagggcaccagcgtcacagtatcctct

SEQ ID NO: 22 - DNA, 324 bp, synthetic construct
  source 1..324: mol_type = other DNA
cagatcctgttgacccaaagtccagctattctttcagcctctttgggcgaacgtgtgactatgacctgcactgcttccagcagcgtgtccagctcctacttgcactggtatcagcagaagcctggttcatcccctaagctgtggatctattccacctccaacctcgcttcaggagtgcctgccagattttccggaggcggaagtggcacttcctactcacttacagtcagcaacatggaggcagaggacgcagctacctactactgccatcagtatcataggtcccctttcactttcgggtccggtaccaagctcgagatcaaa

SEQ ID NO: 23 - protein, 515 aa, synthetic construct
EPHSLRYNLTVLSWDGSVQSGFLTEVHLDGQPFLRCDRQKCRAKPQGQWAEDVLGNKTWDRETRDLTGNGKDLRMTLAHIKDQKEGLHSLQEIRVCEIHEDNSTRSSQHFYYDGELFLSQNLETKEWTMPQSSRAQTLAMNVRNFLKEDAMKTKTHYHAMHADCLQELRRYLKSGVVLRRTVPPMVNVTRSEASEGNITVTCRASGFYPWNITLSWRQDGVSLSHDTQQWGDVLPDGNGTYQTWVATRICQGEEQRFTCYMEHSGNHSTHPVPSGKVLVLQSHWPKSCDKTHTCPPCPAPELLGGPSVFLFPPKPKDTLMISRTPEVTCVVVDVSHEDPEVKFNWYVDGVEVHNAKTKPREEQYNSTYRVVSVLTVLHQDWLNGKEYKCKVSNKALPAPIEKTISKAKGQPREPQVYTLPPSREEMTKNQVSLTCLVKGFYPSDIAVEWESNGQPENNYKTTPPVLDSDGSFFLYSKLTVDKSRWQQGNVFSCSVMHEALHNHYTQKSLSLSPGK

SEQ ID NO: 24 - protein, 339 aa, synthetic construct
VLRRTVPPMVNVTRSEASEGNITVTCRASGFYPWNITLSWRQDGVSLSHDTQQWGDVLPDGNGTYQTWVATRICQGEEQRFTCYMEHSGNHSTHPVPSGKVLVLQSHWPKSCDKTHTCPPCPAPELLGGPSVFLFPPKPKDTLMISRTPEVTCVVVDVSHEDPEVKFNWYVDGVEVHNAKTKPREEQYNSTYRVVSVLTVLHQDWLNGKEYKCKVSNKALPAPIEKTISKAKGQPREPQVYTLPPSREEMTKNQVSLTCLVKGFYPSDIAVEWESNGQPENNYKTTPPVLDSDGSFFLYSKLTVDKSRWQQGNVFSCSVMHEALHNHYTQKSLSLSPGK

SEQ ID NO: 25 - DNA, 1149 bp, synthetic construct
  source 1..1149: mol_type = other DNA
atgggccttggccctgtgtttctgttgcttgctgggatttttccattcgcacctcccggtgccgccgcagagccccacagcttgcggtacaatttgaccgtgctgtcctgggatggcagtgtacaaagcggctttctgaccgaggttcatctggatggacaaccattcctgcgctgcgacagacagaagtgtcgagcaaaaccccagggtcagtgggcagaagatgtactcggcaataagacatgggatcgagaaacaagagacctcacaggaaatggtaaagatctccgcatgacccttgcacacattaaggatcagaaagaaggactgcactccctccaggagattcgagtgtgtgagattcacgaggataacagcacaagaagctcacagcatttttattacgatggagaactgtttctcagccaaaacctggagaccaaagagtggactatgccacagtcctccagagctcagaccctggctatgaatgtccgtaattttttgaaagaggacgcaatgaagaccaagactcactaccatgccatgcacgccgactgcctgcaggagttgagacgatacctcaaatccggggttgtgctcaggcggacagtgcccccaatggtaaacgtgactcggtctgaagcttctgaaggaaacatcacagtcacctgcagagctagcggtttttacccctggaacatcactctctcctggagacaggacggtgtgtccctcagccatgatacccagcagtggggagacgtgctgcccgatggcaacggcacttatcagacttgggtggctactcgaatttgtcaaggagaggagcagcgattcacatgttacatggagcactccgggaatcattcaactcacccagtacccagcggaaaggtccttgtgctgcagagtcattggcagacatttcacgtatccgctgtggcagccgccgcaattttcgtcatcatcattttctatgttcgctgttgtaaaaaaaagacaagcgctgccgaggggcccgaactggtgagcctccaggtgctggaccaacatcccgtgggcaccagcgaccatcgcgatgccacccagcttggcttccagccattgatgtcagacctcggcagcacaggcagcactgagggcgct

SEQ ID NO: 26 - DNA, 1149 bp, synthetic construct
  source 1..1149: mol_type = other DNA
atgggattgggtagggttttgctttttctcgctgtggctttcccctttgcacctcctgctgcagccgcagaaccccatagccttaggtataacctgatggtgctcagtcaagatgaatccgtgcagtccggatttcttgccgagggccatctggatggacaacctttcttgcgttacgataggcagaaacgacgagctaaaccacagggtcagtgggcagaggacgtgctgggagctaagacttgggacaccgagaccgaggatctgactgagaacgggcaggacctgagaaggactctgacacacatcaaggaccagaagggagggttgcactccctgcaggaaatccgcgtgtgtgagattcacgaggactcatcaacccgaggcagtaggcacttttactacgatggagagctgtttctgagtcagaatctggagacacaagagagcactgtgccacagtcatctcgggctcagactctggctatgaacgttaccaatttctggaaagaagatgctatgaaaacaaagacccattatagagctatgcaggccgattgcctgcagaagttgcagcgttatttgaagtctggtgttgctatcaggcggaccgttccccccatggtgaatgtgacttgctccgaggtttccgaaggtaacattactgttacctgtcgagctagctccttctacccacggaacattacattgacatggaggcaggatggcgttagtctgagccataatactcagcagtggggagacgttctgcctgacggaaatggcacataccagacctgggttgccaccagaatccgacagggcgaagagcagaggtttacctgttatatggagcacagcggaaatcatgggactcatcccgtgcctagtgggaaggtgctcgttctccagtctcagcgcactgactttccttacgtgtctgccgctatgccatgcttcgtcatcattatcatcctctgtgtgccatgctgcaagaagaaaacatctgcagccgaggggcctgaacttgtgtccctgcaggttctggaccagcaccctgttggcaccggagatcaccgagacgcagcccaactgggcttccaacctctgatgagcgccactggatctactggttctaccgagggagcc

SEQ ID NO: 27 - DNA, 1098 bp, synthetic construct
  source 1..1098: mol_type = other DNA
atgggccctgggagggttttgctctttctgacctctatttttcccttcgctagaccaggcgctccaacagagctccacagcttgcgctacaacgtgacagttctcagcagggatgggtccgtgcagtccgatttcctcgctgagggccatcttgatagccaactcttcgtccgctacgaccgcgagacacggcgggcaaggccacaaggacagtgggccgaggctgtgctgggcgcaaaaacatgggacactgaaactggcgatctcacagagaatgggaaggacctgcggcgtaccctgactcacattgagggacaaaagggtggcctccacagcttgcaggatatacagaattgtgagatttacgaggacggctctactggaggttccaggcatttttactatgatggggagagatttctgtcccttaatctggccactcaggagtggacagtagcacagtctagccgagcacagactctggccatgaacttctggaaggaagatactatgaaaacaaatacacactaccacgcaatgcaggccgattgcctgaaaaagctgagacgctaccaaaagtccagagtggctgtacgacgcaccgcccctcctatggtgaatgtgacacattccgaggctagtgagggtaatattacagtgacctgccgcgcttctggtttctaccccagaaatatagccttgacctggcgacaggacggtgtttcattgaaccacgacgcccagcagtggggcggcatactgccagaccagaatggcacttaccagacttgggtggccaccaggattcggcagggcgaggaacagcgtttcgcctgctatatggagcatagcggtaatcactctacccatcccgtgcctagcggaaaggtcctggtctttcaatctcagtggctggatattccatacgtgctgggtgtagccgctgccgccgtggccgccgctgccgcaattttcgttattatcctgtacgttctgtgttgcaagaaaaagacttcagccgccgaaggccccgagctcgtgagtctgcgcaccctggatcagcaccccgttggtactggagatcaccgtgacgcaacc

SEQ ID NO: 28 - DNA, 1158 bp, synthetic construct
  source 1..1158: mol_type = other DNA
atgggtctgggaagagtattgctgtttctgggtcgagtcctgctgtttctcgcctccattttctcttttactcgacctcgagccgctgctgagctgcactcactcagatacaacgtgaccgtcttgtctagagatgggtcagtgcagagcgagtttttggcagagggccatttggatggtcagctctttgtgaggtacgatagggaaacacgacgtgctagacctcagggacagtgggcagaggcagtgttgggggaccaggagacagaggacttgaccgagaacgcacaggacctgcgcagaacactgacccacattgaaggccagaagggcggcctgcatagtctgcagaagataaaaatctgcgaaatttatgaggatggctctactggcggattttggcatttttattacgacggggagctgtttctgtcccttaatctggagacacagaagtggacagtagctcagtcatcccgcgctcaaaccctggcaatgaatttctggaaggaggacactatgaaaactaatacacactatagagccatgagggccgattgcttgaaaaaactgtggagataccagaagtctcgggttgctgtgagaaggacagttccccctatggtgaatgtcactcatggggaggcctctgagggcaacataacagtcacatgcagggcttcaggcttttaccctggaaacatcactctgacttggagacaagatggcgtgtccctgagtcacgacgcacaacagtggggcgacgtcctgcctgattggaatggcacctatcagacatgggtcgccacaagaatccgacagggagaggaacagcgttttgcctgttacatggagcatagcggcaatcattccacacatcctgtgccttctggcaagccaccagtgctccagtccgaacggttgaatctgctgtatgtccccgtagcagtggctgttgctgttgtcactgcctttatcattatctgcgttcaccgatgtaaaaagaaaaaaacatcagctgccgagggcccagagttggtatccctcagaactcttgaccaacaccctgtcggaactggggatcatagagatgctacccagctgggattccagcctctcatgagcgctccagggtccaccggatcaactgaaggggcc

SEQ ID NO: 29 - protein, 383 aa, synthetic construct [sequence omitted]

SEQ ID NO: 30 - protein, 366 aa, synthetic construct
MGPGRVLLFLTSIFPFARPGAPTELHSLRYNVTVLSRDGSVQSDFLAEGHLDSQLFVRYDRETRRARPQGQWAEAVLGAKTWDTETGDLTENGKDLRRTLTHIEGQKGGLHSLQDIQNCEIYEDGSTGGSRHFYYDGERFLSLNLATQEWTVAQSSRAQTLAMNFWKEDTMKTNTHYHAMQADCLKKLRRYQKSRVAVRRTAPPMVNVTHSEASEGNITVTCRASGFYPRNIALTWRQDGVSLNHDAQQWGGILPDQNGTYQTWVATRIRQGEEQRFACYMEHSGNHSTHPVPSGKVLVFQSQWLDIPYVLGVAAAAVAAAAAIFVIILYVLCCKKKTSAAEGPELVSLRTLDQHPVGTGDHRDAT

SEQ ID NO: 31 - protein, 386 aa, synthetic construct
MGLGRVLLFLGRVLLFLASIFSFTRPRAAAELHSLRYNVTVLSRDGSVQSEFLAEGHLDGQLFVRYDRETRRARPQGQWAEAVLGDQETEDLTENAQDLRRTLTHIEGQKGGLHSLQKIKICEIYEDGSTGGFWHFYYDGELFLSLNLETQKWTVAQSSRAQTLAMNFWKEDTMKTNTHYRAMRADCLKKLWRYQKSRVAVRRTVPPMVNVTHGEASEGNITVTCRASGFYPGNITLTWRQDGVSLSHDAQQWGDVLPDWNGTYQTWVATRIRQGEEQRFACYMEHSGNHSTHPVPSGKPPVLQSERLNLLYVPVAVAVAVVTAFIIICVHRCKKKKTSAAEGPELVSLRTLDQHPVGTGDHRDATQLGFQPLMSAPGSTGSTEGA

SEQ ID NO: 32 - protein, 375 aa, synthetic construct
IWSAVFLNSLFNQEVQIPLTESYCGPCPKNWICYKNNCYQFFDESKNWYESQASCMSQNASLLKVYSKEDQDLLKLVKSYHWMGLVHIPTNGSWQWEDGSILSPNLLTIIEMQKGDCALYASSFKGYIENCSTPNTYICMQRTVPKSCDKTHTCPPCPAPELLGGPSVFLFPPKPKDTLMISRTPEVTCVVVDVSHEDPEVKFNWYVDGVEVHNAKTKPREEQYNSTYRVVSVLTVLHQDWLNGKEYKCKVSNKALPAPIEKTISKAKGQPREPQVYTLPPSREEMTKNQVSLTCLVKGFYPSDIAVEWESNGQPENNYKTTPPVLDSDGSFFLYSKLTVDKSRWQQGNVFSCSVMHEALHNHYTQKSLSLSPGK

SEQ ID NO: 33 - protein, 336 aa, synthetic construct
RTVPPMVNVTRSEASEGNITVTCRASGFYPWNITLSWRQDGVSLSHDTQQWGDVLPDGNGTYQTWVATRICQGEEQRFTCYMEHSGNHSTHPVPSGKVLVLQSHWPKSCDKTHTCPPCPAPELLGGPSVFLFPPKPKDTLMISRTPEVTCVVVAVSHEDPEVKFNWYVDGVEVHNAKTKPREEQYASTYRVVSVLTVLHQDWLNGKEYKCKVSNKALPAPIEKTISKAKGQPREPQVYTLPPSREEMTKNQVSLTCLVKGFYPSDIAVEWESNGQPENNYKTTPPVLDSDGSFFLYSKLTVDKSRWQQGNVFSCSVMHEALHNHYTQKSLSLSPGK

SEQ ID NO: 34 - protein, 336 aa, synthetic construct
RRVPPMVNVTRSEASEGNITVTCRASSFYPRNITLTWRQDGVSLSHDTQQWGDVLPDGNGTYQTWVATRICQGEEQRFTCYMEHSGNHSTHPVPSGKVLVLQSHWPKSCDKTHTCPPCPAPELLGGPSVFLFPPKPKDTLMISRTPEVTCVVVAVSHEDPEVKFNWYVDGVEVHNAKTKPREEQYASTYRVVSVLTVLHQDWLNGKEYKCKVSNKALPAPIEKTISKAKGQPREPQVYTLPPSREEMTKNQVSLTCLVKGFYPSDIAVEWESNGQPENNYKTTPPVLDSDGSFFLYSKLTVDKSRWQQGNVFSCSVMHEALHNHYTQKSLSLSPGK

SEQ ID NO: 35 - protein, 335 aa, synthetic construct
RTVPPMVNVTCSEVSEGNITVTCRASSFYPRNITLTWRQDGVSLSHNTQQWGDVLPDGNGTYQTWVATRIRQGEEQRFTCYMEHSGNHGTHPVSGKVLVLQSHWPKSCDKTHTCPPCPAPELLGGPSVFLFPPKPKDTLMISRTPEVTCVVVAVSHEDPEVKFNWYVDGVEVHNAKTKPREEQYASTYRVVSVLTVLHQDWLNGKEYKCKVSNKALPAPIEKTISKAKGQPREPQVYTLPPSREEMTKNQVSLTCLVKGFYPSDIAVEWESNGQPENNYKTTPPVLDSDGSFFLYSKLTVDKSRWQQGNVFSCSVMHEALHNHYTQKSLSLSPGK

SEQ ID NO: 36 - protein, 336 aa, synthetic construct
RTVPPMVNVTRSEASEGNITVTCRASSFYPRNIILTWRQDGVSLSHDTQQWGGVLPDGNGTYQTWVATRICRGEEQRFTCYMEHSGNHSTHPVPSGKVLVLQSHWPKSCDKTHTCPPCPAPELLGGPSVFLFPPKPKDTLMISRTPEVTCVVVAVSHEDPEVKFNWYVDGVEVHNAKTKPREEQYASTYRVVSVLTVLHQDWLNGKEYKCKVSNKALPAPIEKTISKAKGQPREPQVYTLPPSREEMTKNQVSLTCLVKGFYPSDIAVEWESNGQPENNYKTTPPVLDSDGSFFLYSKLTVDKSRWQQGNVFSCSVMHEALHNHYTQKSLSLSPGK

SEQ ID NO: 37 - protein, 336 aa, synthetic construct
RTVPPMVNVTCSEVSEGNITVTCRASSFYPRNITLTWRQDGVSLSHNTQQWGDVLPDGNGTYQTWVATRIRQGEEQRFTCYMEHSGNHGTHPVPSGKVLALQSQWPKSCDKTHTCPPCPAPELLGGPSVFLFPPKPKDTLMISRTPEVTCVVVAVSHEDPEVKFNWYVDGVEVHNAKTKPREEQYASTYRVVSVLTVLHQDWLNGKEYKCKVSNKALPAPIEKTISKAKGQPREPQVYTLPPSREEMTKNQVSLTCLVKGFYPSDIAVEWESNGQPENNYKTTPPVLDSDGSFFLYSKLTVDKSRWQQGNVFSCSVMHEALHNHYTQKSLSLSPGK